European Patent Application EP 4 310 188 A1, published January 24, 2024. Title: Gene coding a chimeric receptor against anti-nicotinic acetylcholine receptor auto-antibody. Applicant: DAIICHI SANKYO COMPANY, LIMITED. The sequence listing filed with the application follows.

SEQUENCE LISTING (48 sequences)

SEQ ID NO: 1 - protein, 236 aa, Homo sapiens
SEHETRLVAKLFKDYSSVVRPVEDHRQVVEVTVGLQLIQLINVDEVNQIVTTNVRLKQGDMVDLPRPSCVTLGVPLFSHLQNEQWVDYNLKWNPDDYGGVKKIHIPSEKIWRPDLVLYNNADGDFAIVKFTKVLLQYTGHITWTPPAIFKSYCEIIVTHFPFDEQNCSMKLGTWTYDGSVVAINPESDQPDLSNFMESGEWVIKESRGWKHSVTYSCCPDTPYLDITYHFVMQRLP

SEQ ID NO: 2 - protein, 211 aa, Artificial Sequence
  Native type AChRa211
SEHETRLVAKLFKDYSSVVRPVEDHRQVVEVTVGLQLIQLINVDEVNQIVTTNVRLKQQWVDYNLKWNPDDYGGVKKIHIPSEKIWRPDLVLYNNADGDFAIVKFTKVLLQYTGHITWTPPAIFKSYCEIIVTHFPFDEQNCSMKLGTWTYDGSVVAINPESDQPDLSNFMESGEWVIKESRGWKHSVTYSCCPDTPYLDITYHFVMQRLP

SEQ ID NO: 3 - protein, 211 aa, Artificial Sequence
  AChRa211 with mutation at Xaa8,14,70,72,112 146-159, 192, 193
  at V8mutation (8)..(8): Xaa8 may be any amino acid.
  at D14mutation (14)..(14): Xaa14 may be any amino acid.
  at D70mutation (70)..(70): Xaa70 may be any amino acid.
  at Y72mutation (72)..(72): Xaa72 may be any amino acid.
  at Y112mutation (112)..(112): Xaa112 may be any amino acid.
  at positions 146 to 159mutation (146)..(159): Xaa146 to Xaa159 may be any amino acids.
  misc_feature (192)..(193): Xaa can be any naturally occurring amino acid
SEHETRLXAKLFKXYSSVVRPVEDHRQVVEVTVGLQLIQLINVDEVNQIVTTNVRLKQQWVDYNLKWNPXDXGGVKKIHIPSEKIWRPDLVLYNNADGDFAIVKFTKVLLQXTGHITWTPPAIFKSYCEIIVTHFPFDEQNCSMKXXXXXXXXXXXXXXPESDQPDLSNFMESGEWVIKESRGWKHSVTYSXXPDTPYLDITYHFVMQRLP

SEQ ID NO: 4 - protein, 236 aa, Artificial Sequence
  AChRa236 with mutation at Xaa at position 8, 14,70,72,112, 171-184
  misc_feature (8)..(8): Xaa can be any naturally occurring amino acid
  misc_feature (171)..(184): Xaa can be any naturally occurring amino acid
SEHETRLXAKLFKDYSSVVRPVEDHRQVVEVTVGLQLIQLINVDEVNQIVTTNVRLKQGDMVDLPRPSCVTLGVPLFSHLQNEQWVDYNLKWNPDDYGGVKKIHIPSEKIWRPDLVLYNNADGDFAIVKFTKVLLQYTGHITWTPPAIFKSYCEIIVTHFPFDEQNCSMKXXXXXXXXXXXXXXPESDQPDLSNFMESGEWVIKESRGWKHSVTYSCCPDTPYLDITYHFVMQRLP

SEQ ID NO: 5 - protein, 45 aa, Artificial Sequence
  Linker sequence of CD8a
TTTPAPRPPTPAPTIASQPLSLRPEACRPAAGGAVHTRGLDFACD

SEQ ID NO: 6 - protein, 24 aa, Artificial Sequence
  Transmembrane sequence of CD8a
IYIWAPLAGTCGVLLLSLVITLYC

SEQ ID NO: 7 - protein, 42 aa, Artificial Sequence
  Co-stimulation region of4-1BB
KRGRKKLLYIFKQPFMRPVQTTQEEDGCSCRFPEEEEGGCEL

SEQ ID NO: 8 - protein, 112 aa, Artificial Sequence
  Intracellular signaling region of CD3z
RVKFSRSADAPAYQQGQNQLYNELNLGRREEYDVLDKRRGRDPEMGGKPRRKNPQEGLYNELQKDKMAEAYSEIGMKGERRRGKGHDGLYQGLSTATKDTYDALHMQALPPR

SEQ ID NO: 9 - protein, 21 aa, Artificial Sequence
  Signal peptide sequence of CD8a
MALPVTALLLPLALLLHAARP

SEQ ID NO: 10 - protein, 20 aa, Artificial Sequence
  Signal peptide sequence of AChRa
MEPWPLLLLFSLCSAGLVLG

SEQ ID NO: 11 - protein, 18 aa, Artificial Sequence
  Signal peptide sequence of human immunoglobulin
MDWTWILFLVAAATRVHS

SEQ ID NO: 12 - protein, 501 aa, Homo sapiens
MTPGALLMLLGALGAPLAPGVRGSEAEGRLREKLFSGYDSSVRPAREVGDRVRVSVGLILAQLISLNEKDEEMSTKVYLDLEWTDYRLSWDPAEHDGIDSLRITAESVWLPDVVLLNNNDGNFDVALDISVVVSSDGSVRWQPPGIYRSSCSIQVTYFPFDWQNCTMVFSSYSYDSSEVSLQTGLGPDGQGHQEIHIHEGTFIENGQWEIIHKPSRLIQPPGDPRGGREGQRQEVIFYLIIRRKPLFYLVNVIAPCILITLLAIFVFYLPPDAGEKMGLSIFALLTLTVFLLLLADKVPETSLSVPIIIKYLMFTMVLVTFSVILSVVVLNLHHRSPHTHQMPLWVRQIFIHKLPLYLRLKRPKPERDLMPEPPHCSSPGSGWGRGTDEYFIRKPPSDFLFPKPNRFQPELSAPDLRRFIDGPNRAVALLPELREVVSSISYIARQLQEQEDHDALKEDWQFVAMVVDRLFLWTFIIFTSVGTLVIFLDATYHLPPPDPFP

SEQ ID NO: 13 - protein, 517 aa, Homo sapiens
MEGPVLTLGLLAALAVCGSWGLNEEERLIRHLFQEKGYNKELRPVAHKEESVDVALALTLSNLISLKEVEETLTTNVWIEHGWTDNRLKWNAEEFGNISVLRLPPDMVWLPEIVLENNNDGSFQISYSCNVLVYHYGFVYWLPPAIFRSSCPISVTYFPFDWQNCSLKFSSLKYTAKEITLSLKQDAKENRTYPVEWIIIDPEGFTENGEWEIVHRPARVNVDPRAPLDSPSRQDITFYLIIRRKPLFYIINILVPCVLISFMVNLVFYLPADSGEKTSVAISVLLAQSVFLLLISKRLPATSMAIPLIGKFLLFGMVLVTMVVVICVIVLNIHFRTPSTHVLSEGVKKLFLETLPELLHMSRPAEDGPSPGALVRRSSSLGYISKAEEYFLLKSRSDLMFEKQSERHGLARRLTTARRPPASSEQAQQELFNELKPAVDGANFIVNHMRDQNNYNEEKDSWNRVARTVDRLCLFVVTPVMVVGTAWIFLQGVYNQPPPQPFPGDPYSYNVQDKRFI

SEQ ID NO: 14 - protein, 516 aa, Homo sapiens
MHGGQGPLLLLLLLAVCLGAQGRNQEERLLADLMQNYDPNLRPAERDSDVVNVSLKLTLTNLISLNEREEALTTNVWIEMQWCDYRLRWDPRDYEGLWVLRVPSTMVWRPDIVLENNVDGVFEVALYCNVLVSPDGCIYWLPPAIFRSACSISVTYFPFDWQNCSLIFQSQTYSTNEIDLQLSQEDGQTIEWIFIDPEAFTENGEWAIQHRPAKMLLDPAAPAQEAGHQKVVFYLLIQRKPLFYVINIIAPCVLISSVAILIHFLPAKAGGQKCTVAINVLLAQTVFLFLVAKKVPETSQAVPLISKYLTFLLVVTILIVVNAVVVLNVSLRSPHTHSMARGVRKVFLRLLPQLLRMHVRPLAPAAVQDTQSRLQNGSSGWSITTGEEVALCLPRSELLFQQWQRQGLVAAALEKLEKGPELGLSQFCGSLKQAAPAIQACVEACNLIACARHQQSHFDNGNEEWFLVGRVLDRVCFLAMLSLFICGTAGIFLMAHYNRVPALPFPGDPRPYLPSP

SEQ ID NO: 15 - protein, 20 aa, Artificial Sequence
  Main immunogenic region
DGDFAIVKFTKVLLDYTGHI

SEQ ID NO: 16 - protein, 14 aa, Artificial Sequence
  AChRa211 hydrophobic region 146-159 with mutation G147K
LKTWTYDGSVVAIN

SEQ ID NO: 17 - protein, 14 aa, Artificial Sequence
  AChRa211 hydrophobic region 146-159 with mutation W149K
LGTKTYDGSVVAIN

SEQ ID NO: 18 - protein, 14 aa, Artificial Sequence
  AChRa211 hydrophobic region 146-159 with mutation Y151K
LGTWTKDGSVVAIN

SEQ ID NO: 19 - protein, 14 aa, Artificial Sequence
  AChRa211 hydrophobic region 146-159 with mutation G153K
LGTWTYDKSVVAIN

SEQ ID NO: 20 - protein, 14 aa, Artificial Sequence
  AChRa211 hydrophobic region 146-159 with mutation V155K
LGTWTYDGSKVAIN

SEQ ID NO: 21 - protein, 14 aa, Artificial Sequence
  AChRa211 hydrophobic region 146-159 with mutation A157K
LGTWTYDGSVVKIN

SEQ ID NO: 22 - protein, 14 aa, Artificial Sequence
  AChRa211 hydrophobic region 146-159 with mutation N159K
LGTWTYDGSVVAIK

SEQ ID NO: 23 - protein, 14 aa, Artificial Sequence
  AChRa211 hydrophobic region 146-159 with mutations W149R, V155K
LGTRTYDGSKVAIN

SEQ ID NO: 24 - protein, 594 aa, Artificial Sequence
  mAb35
MALPVTALLLPLALLLHAARPSNIQLTQSPSLLSASVGDRVTLTCKGSQNIDNYLAWYQQKLGEAPKLLIYKTNSLQTGIPSRFSGSGSGTDYTLTISSLHSEDLATYYCYQYINGYTFGTGTKLELKRGGGGSGGGGSGGGGSQVQLKESGPGLVQPSETLSLTCTVSGFSLTSYSVSWLRQPSGKGPEWMGRMWDDGGTVYNSGLKSRLSISRDTSKNQVFLKMNSLQTDDTGTYYCTRDERIRAINWFAYWGQGTLVTVSSASTKGPSVFPLAPSSKSTSGGTAALGCLVKDYFPEPVTVSWNSGALTSGVHTFPAVLQSSGLYSLSSVVTVPSSSLGTQTYICNVNHKPSNTKVDKKVEPKSCDKTHTCPPCPAPELLGGPSVFLFPPKPKDTLMISRTPEVTCVVVDVSHEDPEVKFNWYVDGVEVHNAKTKPREEQYNSTYRVVSVLTVLHQDWLNGKEYKCKVSNKALPAPIEKTISKAKGQPREPQVYTLPPSRDELTKNQVSLTCLVKGFYPSDIAVEWESNGQPENNYKTTPPVLDSDGSFFLYSKLTVDKSRWQQGNVFSCSVMHEALHNHYTQKSLSLSPGK

SEQ ID NO: 25 - protein, 41 aa, Artificial Sequence
  CD28 co-stimulation region
RSKRSRLLHSDYMNMTPRRPGPTRKHYQPYAPPRDFAAYRS

SEQ ID NO: 26 - protein, 58 aa, Artificial Sequence
  GITR co-stimulation region
QLGLHIWQLRSQCMWPRETQLLLEVPPSTEDARSCQFPEEERGERSAEEKGRLGDLWV

SEQ ID NO: 27 - protein, 58 aa, Artificial Sequence; identical to SEQ ID NO: 26
  TNFR2 co-stimulation region

SEQ ID NO: 28 - protein, 197 aa, Artificial Sequence
  DR3 co-stimulation region
TYTYRHCWPHKPLVTADEAGMEALTPPPATHLSPLDSAHTLLAPPDSSEKICTVQLVGNSWTPGYPETQEALCPQVTWSWDQLPSRALGPAAAPTLSPESPAGSPAMMLQPGPQLYDVMDAVPARRWKEFVRTLGLREAEIEAVEVEIGRFRDQQYEMLKRWRQQQPAGLGAVYAALERMGLDGCVEDLRSRLQRGP

SEQ ID NO: 29 - protein, 189 aa, Artificial Sequence
  CD30 co-stimulation region
CHRRACRKRIRQKLHLCYPVQTSQPKLELVDSRPRRSSTQLRSGASVTEPVAEERGLMSQPLMETCHSVGAAYLESLPLQDASPAGGPSSPRDLPEPRVSTEHTNNKIEKIYIMKADTVIVGTVKAELPEGRGLAGPAEPELEEELEADHTPHYPEQETEPPLGSCSDVMLSVEEEGKEDPLPTAASGK

SEQ ID NO: 30 - protein, 60 aa, Artificial Sequence
  HVEM co-stimulation region
CVKRRKPRGDVVKVIVSVQRKRQEAEGEATVIEALQAPPDVTTVAVEETIPSFTGRSPNH

SEQ ID NO: 31 - protein, 47 aa, Artificial Sequence
  CD27 co-stimulation region
RRKYRSNKGESPVEPAEPCRYSCPREEEGSTIPIQEDYRKPEPACSP

SEQ ID NO: 32 - protein, 37 aa, Artificial Sequence
  ox40 co-stimulation region
RRDQRLPPDAHKPPGGGSFRTPIQEEQADAHSTLAKI

SEQ ID NO: 33 - protein, 791 aa, Artificial Sequence
  divalent mAb35
MAVLVLLLCLVTLPSCVLAQVQLKESGPGLVQPSETLSLTCTVSGFSLTSYSVSWLRQPSGKGPEWMGRMWDDGGTVYNSGLKSRLSISRDTSKNQVFLKMNSLQTDDTGTYYCTRDERIRAINWFAYWGQGTLVTVSSASTKGPSVFPLAPSSKSTSGGTAALGCLVKDYFPEPVTVSWNSGALTSGVHTFPAVLQSSGLYSLSSVVTVPSSSLGTQTYICNVNHKPSNTKVDKKVEPKSCDKTHTCPPCPAPELLGGPSVFLFPPKPKDTLMISRTPEVTCVVVDVSHEDPEVKFNWYVDGVEVHNAKTKPREEQYNSTYRVVSVLTVLHQDWLNGKEYKCKVSNKALPAPIEKTISKAKGQPREPQVYTLPPSRDELTKNQVSLTCLVKGFYPSDIAVEWESNGQPENNYKTTPPVLDSDGSFFLYSKLTVDKSRWQQGNVFSCSVMHEALHNHYTQKSLSLSPELQLEESCAEAQDGELDGLWTTITIFITLFLLSVCYSATVTFFKVKWIFSSVVDLKQTIIPDYRNMIGQGAGSGEGRGSLLTCGDVEENPGPMAPAQLLGLLLLWLPAMRCNIQLTQSPSLLSASVGDRVTLTCKGSQNIDNYLAWYQQKLGEAPKLLIYKTNSLQTGIPSRFSGSGSGTDYTLTISSLHSEDLATYYCYQYINGYTFGTGTKLELKRTVAAPSVFIFPPSDEQLKSGTASVVCLLNNFYPREAKVQWKVDNALQSGNSQESVTEQDSKDSTYSLSSTLTLSKADYEKHKVYACEVTHQGLSSPVTKSFNRGEC

SEQ ID NO: 34 - protein, 476 aa, Artificial Sequence
  CD79a/CD79b
MPGGPGVLQALPATIFLLFLLSAVYLGPGCQALWMHKVPASLMVSLGEDAHFQCPHNSSNNANVTWWRVLHGNYTWPPEFLGPGEDPNGTLIIQNVNKSHGGIYVCRVQEGNESYQQSCGTYLRVRQPPPRPFLDMGEGTKNRIITAEGIILLFCAVVPGTLLLFRKRWQNEKLGLDAGDEYEDENLYEGLNLDDCSMYEDISRGLQGTYQDVGSLNIGDVQLEKPGSGEGRGSLLTCGDVEENPGPMARLALSPVPSHWMVALLLLLSAEPVPAARSEDRYRNPKGSACSRIWQSPRFIARKRGFTVKMHCYMNSASGNVSWLWKQEMDENPQQLKLEKGRMEESQNESLATLTIQGIRFEDNGIYFCQQKCNNTSEVYQGCGTELRVMGFSTLAQLKQRNTLKDGIIMIQTLLIILFIIVPIFLLLDKDDSKAGMEEDHTYEGLDIDQTATYEDIVTLRTGEVKWSVGEHPGQE

SEQ ID NO: 35 - protein, 469 aa, Artificial Sequence
  mAb35 hIgG1
MAVLVLLLCLVTLPSCVLAQVQLKESGPGLVQPSETLSLTCTVSGFSLTSYSVSWLRQPSGKGPEWMGRMWDDGGTVYNSGLKSRLSISRDTSKNQVFLKMNSLQTDDTGTYYCTRDERIRAINWFAYWGQGTLVTVSSASTKGPSVFPLAPSSKSTSGGTAALGCLVKDYFPEPVTVSWNSGALTSGVHTFPAVLQSSGLYSLSSVVTVPSSSLGTQTYICNVNHKPSNTKVDKKVEPKSCDKTHTCPPCPAPELLGGPSVFLFPPKPKDTLMISRTPEVTCVVVDVSHEDPEVKFNWYVDGVEVHNAKTKPREEQYNSTYRVVSVLTVLHQDWLNGKEYKCKVSNKALPAPIEKTISKAKGQPREPQVYTLPPSRDELTKNQVSLTCLVKGFYPSDIAVEWESNGQPENNYKTTPPVLDSDGSFFLYSKLTVDKSRWQQGNVFSCSVMHEALHNHYTQKSLSLSPGK

SEQ ID NO: 36 - protein, 232 aa, Artificial Sequence
  mAb35 hIgGk
MAPAQLLGLLLLWLPAMRCNIQLTQSPSLLSASVGDRVTLTCKGSQNIDNYLAWYQQKLGEAPKLLIYKTNSLQTGIPSRFSGSGSGTDYTLTISSLHSEDLATYYCYQYINGYTFGTGTKLELKRTVAAPSVFIFPPSDEQLKSGTASVVCLLNNFYPREAKVQWKVDNALQSGNSQESVTEQDSKDSTYSLSSTLTLSKADYEKHKVYACEVTHQGLSSPVTKSFNRGEC

SEQ ID NO: 37 - protein, 27 aa, Artificial Sequence
  CD28 transmembrane region
FWVLVVVGGVLACYSLLVTVAFIIFWV

SEQ ID NO: 38 - protein, 24 aa, Artificial Sequence
  AChRa transmembrane region
LYFIVNVIIPCLLFSFLTGLVFYL

SEQ ID NO: 39 - protein, 45 aa, Artificial Sequence
  CD8a linker optionally with mutation at Xaa27 and/or Xaa44
  mutation (27)..(27): Xaa27 is Cys or Ser
  mutation (44)..(44): Xaa44 is Cys or Ser
TTTPAPRPPTPAPTIASQPLSLRPEAXRPAAGGAVHTRGLDFAXD

SEQ ID NO: 40 - protein, 39 aa, Artificial Sequence
  CD28 linker optionally with mutation at Xaa28
  mutation (28)..(28): Xaa28 is Cys or Ser
IEVMYPPPYLDNEKSNGTIIHVKGKHLXPSPLFPGPSKP

SEQ ID NO: 41 - protein, 14 aa, Artificial Sequence
  Artificial flexible linker sequence
ASGGGGSGGGGSSG

SEQ ID NO: 42 - protein, 211 aa, Artificial Sequence
  AChRa211 in which D14, W149 and or V155 may be mutated.
  Xaa14_mutation (14)..(14): Xaa14 may be any amino acids, preferably Asp, Ala or Gly.
  Xaa149_mutation (149)..(149): Xaa149 may be any amino acids, preferably Trp, Arg, Ala, Lys, Asp, Ser, Gly, Asn, Ile, Phe, Met or Pro.
  Xaa155_mutation (155)..(155): Xaa155 may be any amino acids, preferably Val, Arg, Lys, Asp, Ser, Gly, Asn, Ile, Phe, Met or Pro.
SEHETRLVAKLFKXYSSVVRPVEDHRQVVEVTVGLQLIQLINVDEVNQIVTTNVRLKQQWVDYNLKWNPDDYGGVKKIHIPSEKIWRPDLVLYNNADGDFAIVKFTKVLLQYTGHITWTPPAIFKSYCEIIVTHFPFDEQNCSMKLGTXTYDGSXVAINPESDQPDLSNFMESGEWVIKESRGWKHSVTYSCCPDTPYLDITYHFVMQRLP

SEQ ID NO: 43 - protein, 434 aa, Artificial Sequence
  AChRa211/W149R/V155K>45aa>4-1BB
SEHETRLVAKLFKDYSSVVRPVEDHRQVVEVTVGLQLIQLINVDEVNQIVTTNVRLKQQWVDYNLKWNPDDYGGVKKIHIPSEKIWRPDLVLYNNADGDFAIVKFTKVLLQYTGHITWTPPAIFKSYCEIIVTHFPFDEQNCSMKLGTRTYDGSKVAINPESDQPDLSNFMESGEWVIKESRGWKHSVTYSCCPDTPYLDITYHFVMQRLPTTTPAPRPPTPAPTIASQPLSLRPEACRPAAGGAVHTRGLDFACDIYIWAPLAGTCGVLLLSLVITLYCKRGRKKLLYIFKQPFMRPVQTTQEEDGCSCRFPEEEEGGCELRVKFSRSADAPAYQQGQNQLYNELNLGRREEYDVLDKRRGRDPEMGGKPRRKNPQEGLYNELQKDKMAEAYSEIGMKGERRRGKGHDGLYQGLSTATKDTYDALHMQALPPR

SEQ ID NO: 44 - protein, 393 aa, Artificial Sequence
  AChRa211/W149R/V155K>4aa>4-1BB
SEHETRLVAKLFKDYSSVVRPVEDHRQVVEVTVGLQLIQLINVDEVNQIVTTNVRLKQQWVDYNLKWNPDDYGGVKKIHIPSEKIWRPDLVLYNNADGDFAIVKFTKVLLQYTGHITWTPPAIFKSYCEIIVTHFPFDEQNCSMKLGTRTYDGSKVAINPESDQPDLSNFMESGEWVIKESRGWKHSVTYSCCPDTPYLDITYHFVMQRLPGSSGIYIWAPLAGTCGVLLLSLVITLYCKRGRKKLLYIFKQPFMRPVQTTQEEDGCSCRFPEEEEGGCELRVKFSRSADAPAYQQGQNQLYNELNLGRREEYDVLDKRRGRDPEMGGKPRRKNPQEGLYNELQKDKMAEAYSEIGMKGERRRGKGHDGLYQGLSTATKDTYDALHMQALPPR

SEQ ID NO: 45 - protein, 434 aa, Artificial Sequence
  AChRa211/D14G/W149R/V155K>45aa> 4-1BB
SEHETRLVAKLFKGYSSVVRPVEDHRQVVEVTVGLQLIQLINVDEVNQIVTTNVRLKQQWVDYNLKWNPDDYGGVKKIHIPSEKIWRPDLVLYNNADGDFAIVKFTKVLLQYTGHITWTPPAIFKSYCEIIVTHFPFDEQNCSMKLGTRTYDGSKVAINPESDQPDLSNFMESGEWVIKESRGWKHSVTYSCCPDTPYLDITYHFVMQRLPTTTPAPRPPTPAPTIASQPLSLRPEACRPAAGGAVHTRGLDFACDIYIWAPLAGTCGVLLLSLVITLYCKRGRKKLLYIFKQPFMRPVQTTQEEDGCSCRFPEEEEGGCELRVKFSRSADAPAYQQGQNQLYNELNLGRREEYDVLDKRRGRDPEMGGKPRRKNPQEGLYNELQKDKMAEAYSEIGMKGERRRGKGHDGLYQGLSTATKDTYDALHMQALPPR

SEQ ID NO: 46 - protein, 429 aa, Artificial Sequence
  AChRa211/W149R/V155K >45aa>OX40
SEHETRLVAKLFKDYSSVVRPVEDHRQVVEVTVGLQLIQLINVDEVNQIVTTNVRLKQQWVDYNLKWNPDDYGGVKKIHIPSEKIWRPDLVLYNNADGDFAIVKFTKVLLQYTGHITWTPPAIFKSYCEIIVTHFPFDEQNCSMKLGTRTYDGSKVAINPESDQPDLSNFMESGEWVIKESRGWKHSVTYSCCPDTPYLDITYHFVMQRLPTTTPAPRPPTPAPTIASQPLSLRPEACRPAAGGAVHTRGLDFACDIYIWAPLAGTCGVLLLSLVITLYCRRDQRLPPDAHKPPGGGSFRTPIQEEQADAHSTLAKIRVKFSRSADAPAYQQGQNQLYNELNLGRREEYDVLDKRRGRDPEMGGKPRRKNPQEGLYNELQKDKMAEAYSEIGMKGERRRGKGHDGLYQGLSTATKDTYDALHMQALPPR

SEQ ID NO: 47 - protein, 398 aa, Artificial Sequence
  AChRa211/W149R/V155K >14aa>OX40
SEHETRLVAKLFKDYSSVVRPVEDHRQVVEVTVGLQLIQLINVDEVNQIVTTNVRLKQQWVDYNLKWNPDDYGGVKKIHIPSEKIWRPDLVLYNNADGDFAIVKFTKVLLQYTGHITWTPPAIFKSYCEIIVTHFPFDEQNCSMKLGTRTYDGSKVAINPESDQPDLSNFMESGEWVIKESRGWKHSVTYSCCPDTPYLDITYHFVMQRLPGGAVHTRGLDFACDIYIWAPLAGTCGVLLLSLVITLYCRRDQRLPPDAHKPPGGGSFRTPIQEEQADAHSTLAKIRVKFSRSADAPAYQQGQNQLYNELNLGRREEYDVLDKRRGRDPEMGGKPRRKNPQEGLYNELQKDKMAEAYSEIGMKGERRRGKGHDGLYQGLSTATKDTYDALHMQALPPR

SEQ ID NO: 48 - protein, 32 aa, Artificial Sequence
  Amino acid sequence containing signal peptide and FLAG tag peptide
MALPVTALLLPLALLLHAARPDYKDDDDKGSG